European Patent Specification EP 3 642 333 B1, published September 10, 2025. Title: Embryonic neural border stem cells. Applicant: HI-STEM gGmbH. The sequence listing filed with the application follows.

SEQUENCE LISTING (105 sequences)

SEQ ID NO: 1 - DNA, 12099 bp, artificial sequence
  artificial vector
tggaagggctaattcactcccaaagaagacaagatatccttgatctgtggatctaccacacacaaggctacttccctgattagcagaactacacaccagggccaggggtcagatatccactgacctttggatggtgctacaagctagtaccagttgagccagataaggtagaagaggccaataaaggagagaacaccagcttgttacaccctgtgagcctgcatgggatggatgacccggagagagaagtgttagagtggaggtttgacagccgcctagcatttcatcacgtggcccgagagctgcatccggagtacttcaagaactgctgatatcgagcttgctacaagggactttccgctggggactttccagggaggcgtggcctgggcgggactggggagtggcgagccctcagatcctgcatataagcagctgctttttgcctgtactgggtctctctggttagaccagatctgagcctgggagctctctggctaactagggaacccactgcttaagcctcaataaagcttgccttgagtgcttcaagtagtgtgtgcccgtctgttgtgtgactctggtaactagagatccctcagacccttttagtcagtgtggaaaatctctagcagtggcgcccgaacagggacttgaaagcgaaagggaaaccagaggagctctctcgacgcaggactcggcttgctgaagcgcgcacggcaagaggcgaggggcggcgactggtgagtacgccaaaaattttgactagcggaggctagaaggagagagatgggtgcgagagcgtcagtattaagcgggggagaattagatcgcgatgggaaaaaattcggttaaggccagggggaaagaaaaaatataaattaaaacatatagtatgggcaagcagggagctagaacgattcgcagttaatcctggcctgttagaaacatcagaaggctgtagacaaatactgggacagctacaaccatcccttcagacaggatcagaagaacttagatcattatataatacagtagcaaccctctattgtgtgcatcaaaggatagagataaaagacaccaaggaagctttagacaagatagaggaagagcaaaacaaaagtaagaccaccgcacagcaagcggccggccgctgatcttcagacctggaggaggagatatgagggacaattggagaagtgaattatataaatataaagtagtaaaaattgaaccattaggagtagcacccaccaaggcaaagagaagagtggtgcagagagaaaaaagagcagtgggaataggagctttgttccttgggttcttgggagcagcaggaagcactatgggcgcagcgtcaatgacgctgacggtacaggccagacaattattgtctggtatagtgcagcagcagaacaatttgctgagggctattgaggcgcaacagcatctgttgcaactcacagtctggggcatcaagcagctccaggcaagaatcctggctgtggaaagatacctaaaggatcaacagctcctggggatttggggttgctctggaaaactcatttgcaccactgctgtgccttggaatgctagttggagtaataaatctctggaacagatttggaatcacacgacctggatggagtgggacagagaaattaacaattacacaagcttaatacactccttaattgaagaatcgcaaaaccagcaagaaaagaatgaacaagaattattggaattagataaatgggcaagtttgtggaattggtttaacataacaaattggctgtggtatataaaattattcataatgatagtaggaggcttggtaggtttaagaatagtttttgctgtactttctatagtgaatagagttaggcagggatattcaccattatcgtttcagacccacctcccaaccccgaggggacccgacaggcccgaaggaatagaagaagaaggtggagagagagacagagacagatccattcgattagtgaacggatctcgacggtatcgccgaattcacaaatggcagtattcatccacaattttaaaagaaaaggggggattggggggtacagtgcaggggaaagaatagtagacataatagcaacagacatacaaactaaagaattacaaaaacaaattacaaaaattcaaaattttcgggtttattacagggacagcagagatccagtttggactagtccacaccctaactgacacactcgagtttaccactccctatcagtgatagagaaaagtgaaagtcgagtttaccactccctatcagtgatagagaaaagtgaaagtcgagtttaccactccctatcagtgatagagaaaagtgaaagtcgagtttaccactccctatcagtgatagagaaaagtgaaagtcgagtttaccactccctatcagtgatagagaaaagtgaaagtcgagtttaccactccctatcagtgatagagaaaagtgaaagtcgagtttaccactccctatcagtgatagagaaaagtgaaagtcgagctcggtacccgggtcgaggtaggcgtgtacggtgggaggcctatataagcagagctcgtttagtgaaccgtcagatcgcctggagacgccatccacgctgttttgacctccatagaagacaccgggaccgatccagcctgcggccgccatggcgaccgcagcgtctaaccactacagcctgctcacctccagcgcctccatcgtgcacgccgagccgcccggcggcatgcagcagggcgcggggggctaccgcgaagcgcagagcctggtgcagggcgactacggcgctctgcagagcaacggacacccgctcagccacgctcaccagtggatcaccgcgctgtcccacggcggcggcggcgggggcggtggcggcggcggggggggcgggggcggcggcgggggcggcggcgacggctccccgtggtccaccagccccctgggccagccggacatcaagccctcggtggtggtgcagcagggcggccgcggagacgagctgcacgggccaggcgccctgcagcagcagcatcagcagcagcaacagcaacagcagcagcaacagcagcaacagcagcagcagcagcagcaacagcggccgccgcatctggtgcaccacgccgctaaccaccacccgggacccggggcatggcggagcgcggcggctgcagcgcacctcccaccctccatgggagcgtccaacggcggcttgctctactcgcagcccagcttcacggtgaacggcatgctgggcgccggcgggcagccggccggtctgcaccaccacggcctgcgggacgcgcacgacgagccacaccatgccgaccaccacccgcacccgcactcgcacccacaccagcagccgccgcccccgccgcccccgcagggtccgcctggccacccaggcgcgcaccacgacccgcactcggacgaggacacgccgacctcggacgacctggagcagttcgccaagcagttcaagcagcggcggatcaaactgggatttacccaagcggacgtggggctggctctgggcaccctgtatggcaacgtgttctcgcagaccaccatctgcaggtttgaggccctgcagctgagcttcaagaacatgtgcaagctgaagcctttgttgaacaagtggttggaggaggcggactcgtcctcgggcagccccacgagcatagacaagatcgcagcgcaagggcgcaagcggaaaaagcggacctccatcgaggtgagcgtcaagggggctctggagagccatttcctcaaatgccccaagccctcggcccaggagatcacctccctcgcggacagcttacagctggagaaggaggtggtgagagtttggttttgtaacaggagacagaaagagaaaaggatgacccctcccggagggactctgccgggcgccgaggatgtgtacggggggagtagggacactccaccacaccacggggtgcagacgcccgtccagggaagtggcgtgaaacagactttgaattttgaccttctcaagttggcgggagacgtggagtccaacccagggcccatggctgtcagcgacgctctgctcccgtccttctccacgttcgcgtccggcccggcgggaagggagaagacactgcgtccagcaggtgccccgactaaccgttggcgtgaggaactctctcacatgaagcgacttcccccacttcccggccgcccctacgacctggcggcgacggtggccacagacctggagagtggcggagctggtgcagcttgcagcagtaacaacccggccctcctagcccggagggagaccgaggagttcaacgacctcctggacctagactttatcctttccaactcgctaacccaccaggaatcggtggccgccaccgtgaccacctcggcgtcagcttcatcctcgtcttccccagcgagcagcggccctgccagcgcgccctccacctgcagcttcagctatccgatccgggccgggggtgacccgggcgtggctgccagcaacacaggtggagggctcctctacagccgagaatctgcgccacctcccacggcccccttcaacctggcggacatcaatgacgtgagcccctcgggcggcttcgtggctgagctcctgcggccggagttggacccagtatacattccgccacagcagcctcagccgccaggtggcgggctgatgggcaagtttgtgctgaaggcgtctctgaccacccctggcagcgagtacagcagcccttcggtcatcagtgttagcaaaggaagcccagacggcagccaccccgtggtagtggcgccctacagcggtggcccgccgcgcatgtgccccaagattaagcaagaggcggtcccgtcctgcacggtcagccggtccctagaggcccatttgagcgctggaccccagctcagcaacggccaccggcccaacacacacgacttccccctggggcggcagctccccaccaggactacccctacactgagtcccgaggaactgctgaacagcagggactgtcaccctggcctgcctcttcccccaggattccatccccatccggggcccaactaccctcctttcctgccagaccagatgcagtcacaagtcccctctctccattatcaagagctcatgccaccgggttcctgcctgccagaggagcccaagccaaagaggggaagaaggtcgtggccccggaaaagaacagccacccacacttgtgactatgcaggctgtggcaaaacctataccaagagttctcatctcaaggcacacctgcgaactcacacaggcgagaaaccttaccactgtgactgggacggctgtgggtggaaattcgcccgctccgatgaactgaccaggcactaccgcaaacacacagggcaccggccctttcagtgccagaagtgtgacagggccttttccaggtcggaccaccttgccttacacatgaagaggcacttttaaagatccctcccccccccctaacgttactggccgaagccgcttggaataaggccggtgtgcgtttgtctatatgttattttccaccatattgccgtcttttggcaatgtgagggcccggaaacctggccctgtcttcttgacgagcattcctaggggtctttcccctctcgccaaaggaatgcaaggtctgttgaatgtcgtgaaggaagcagttcctctggaagcttcttgaagacaaacaacgtctgtagcgaccctttgcaggcagcggaaccccccacctggcgacaggtgcctctgcggccaaaagccacgtgtataagatacacctgcaaaggcggcacaaccccagtgccacgttgtgagttggatagttgtggaaagagtcaaatggctctcctcaagcgtattcaacaaggggctgaaggatgcccagaaggtaccccattgtatgggatctgatctggggcctcggtgcacatgctttacatgtgtttagtcgaggttaaaaaaacgtctaggccccccgaaccacggggacgtggttttcctttgaaaaacacgatgataatatggccacacatatgatgtataacatgatggagacggagctgaagccgccgggcccgcagcaagcttcggggggcggcggcggaggaggcaacgccacggcggcggcgaccggcggcaaccagaagaacagcccggaccgcgtcaagaggcccatgaacgccttcatggtatggtcccgggggcagcggcgtaagatggcccaggagaaccccaagatgcacaactcggagatcagcaagcgcctgggcgcggagtggaaacttttgtccgagaccgagaagcggccgttcatcgacgaggccaagcggctgcgcgctctgcacatgaaggagcacccggattataaataccggccgcggcggaaaaccaagacgctcatgaagaaggataagtacacgcttcccggaggcttgctggcccccggcgggaacagcatggcgagcggggttggggtgggcgccggcctgggtgcgggcgtgaaccagcgcatggacagctacgcgcacatgaacggctggagcaacggcagctacagcatgatgcaggagcagctgggctacccgcagcacccgggcctcaacgctcacggcgcggcacagatgcaaccgatgcaccgctacgacgtcagcgccctgcagtacaactccatgaccagctcgcagacctacatgaacggctcgcccacctacagcatgtcctactcgcagcagggcacccccggtatggcgctgggctccatgggctctgtggtcaagtccgaggccagctccagcccccccgtggttacctcttcctcccactccagggcgccctgccaggccggggacctccgggacatgatcagcatgtacctccccggcgccgaggtgccggagcccgctgcgcccagtagactgcacatggcccagcactaccagagcggcccggtgcccggcacggccattaacggcacactgcccctgtcgcacatgggtagtgggcaatgtactaactacgctttgttgaaactcgctggcgatgttgaaagtaaccccggtcctatgacgatgctcctggacggaggcccgcagttccctgggttgggagtgggcagcttcggtgctccgcgccaccacgagatgcccaaccgcgagcctgcaggcatgggattgaatcccttcggggactcaacccacgctgcggccgccgccgctgccgccgctgccttcaagctgagcccagccaccgctcacgatctgtcttcgggccagagctcagcgttcacaccgcagggttcaggttatgccaatgccctgggccaccatcaccaccaccatcaccaccatcacgccagccaggtgcccacctacggcggcgctgcctccgccgctttcaactccacgcgcgactttctgttccgtcagcgcggttctgggctcagcgaggcagcctccgggggcgggcagcacgggcttttcgctggctcggcgagcagtcttcacgctccagctggtattcctgagcctcctagctacttgctctttcctgggcttcatgagcagggcgctgggcacccgtcgcccacagggcacgtggacaacaaccaggtccatctggggctgcgcggggagctatttggccgtgcagacccataccgccccgtggctagcccgcgcacggacccctacgcggccagtgcgcagttccctaactatagccccatgaacatgaacatgggcgtgaacgtggcggcccaccacgggccgggcgccttcttccgttacatgcggcagcccatcaagcaggagctgtcctgtaagtggatcgaggaggctcagctgagccggcccaagaagagctgcgaccggaccttcagcaccatgcatgagttggttacgcatgttaccatggagcatgtggggggcccggagcagaacaaccacgtctgctattgggaggaatgtccccgcgaaggcaagtccttcaaggcgaagtacaaactggtcaaccatatccgagtgcacactggcgagaaacccttcccgtgtcccttcccgggctgcgggaagatttttgcccgctctgagaacctcaagatccacaagaggacccatacaggtgagaaacctttcaaatgtgaattcgaaggctgtgacagacggtttgccaacagcagcgaccgcaagaagcacatgcatgtgcacacctcggacaagccctatatctgtaaagtgtgcgacaagtcctacacacacccgagctccctgcgcaaacacatgaaggttcatgaatctcaagggtcagattcctcccctgctgccagttcaggctatgaatcttccactccacccgctatagcttctgcaaacagtaaagataccactaaaaccccttctgcagttcaaactagcaccagccacaaccctggacttcctcccaattttaacgaatggtacgtctgaatcgatagatcctaatcaacctctggattacaaaatttgtgaaagattgactggtattcttaactatgttgctccttttacgctatgtggatacgctgctttaatgcctttgtatcatgctattgcttcccgtatggctttcattttctcctccttgtataaatcctggttgctgtctctttatgaggagttgtggcccgttgtcaggcaacgtggcgtggtgtgcactgtgtttgctgacgcaacccccactggttggggcattgccaccacctgtcagctcctttccgggactttcgctttccccctccctattgccacggcggaactcatcgccgcctgccttgcccgctgctggacaggggctcggctgttgggcactgacaattccgtggtgttgtcggggaaatcatcgtcctttccttggctgctcgcctgtgttgccacctggattctgcgcgggacgtccttctgctacgtcccttcggccctcaatccagcggaccttccttcccgcggcctgctgccggctctgcggcctcttccgcgtcttcgccttcgccctcagacgagtcggatctccctttgggccgcctccccgcctggtacctttaagaccaatgacttacaaggcagctgtagatcttagccactttttaaaagaaaaggggggactggaagggctaattcactcccaacgaagacaagatcacctgcaggacaggcgcgccctgctttttgcttgtactgggtctctctggttagaccagatctgagcctgggagctctctggctaactagggaacccactgcttaagcctcaataaagcttgccttgagtgcttcaagtagtgtgtgcccgtctgttgtgtgactctggtaactagagatccctcagacccttttagtcagtgtggaaaatctctagcacccgggcgattaaggaaagggctagatcattcttgaagacgaaagggcctcgtgatacgcctatttttataggttaatgtcatgataataatggtttcttagacgtcaggtggcacttttcggggaaatgtgcgcggaacccctatttgtttatttttctaaatacattcaaatatgtatccgctcatgagacaataaccctgataaatgcttcaataatattgaaaaaggaagagtatgagtattcaacatttccgtgtcgcccttattcccttttttgcggcattttgccttcctgtttttgctcacccagaaacgctggtgaaagtaaaagatgctgaagatcagttgggtgcacgagtgggttacatcgaactggatctcaacagcggtaagatccttgagagttttcgccccgaagaacgttttccaatgatgagcacttttaaagttctgctatgtggcgcggtattatcccgtgttgacgccgggcaagagcaactcggtcgccgcatacactattctcagaatgacttggttgagtactcaccagtcacagaaaagcatcttacggatggcatgacagtaagagaattatgcagtgctgccataaccatgagtgataacactgcggccaacttacttctgacaacgatcggaggaccgaaggagctaaccgcttttttgcacaacatgggggatcatgtaactcgccttgatcgttgggaaccggagctgaatgaagccataccaaacgacgagcgtgacaccacgatgcctgtagcaatggcaacaacgttgcgcaaactattaactggcgaactacttactctagcttcccggcaacaattaatagactggatggaggcggataaagttgcaggaccacttctgcgctcggcccttccggctggctggtttattgctgataaatctggagccggtgagcgtgggtctcgcggtatcattgcagcactggggccagatggtaagccctcccgtatcgtagttatctacacgacggggagtcaggcaactatggatgaacgaaatagacagatcgctgagataggtgcctcactgattaagcattggtaactgtcagaccaagtttactcatatatactttagattgatttaaaacttcatttttaatttaaaaggatctaggtgaagatcctttttgataatctcatgaccaaaatcccttaacgtgagttttcgttccactgagcgtcagaccccgtagaaaagatcaaaggatcttcttgagatcctttttttctgcgcgtaatctgctgcttgcaaacaaaaaaaccaccgctaccagcggtggtttgtttgccggatcaagagctaccaactctttttccgaaggtaactggcttcagcagagcgcagataccaaatactgttcttctagtgtagccgtagttaggccaccacttcaagaactctgtagcaccgcctacatacctcgctctgctaatcctgttaccagtggctgctgccagtggcgataagtcgtgtcttaccgggttggactcaagacgatagttaccggataaggcgcagcggtcgggctgaacggggggttcgtgcacacagcccagcttggagcgaacgacctacaccgaactgagatacctacagcgtgagctatgagaaagcgccacgcttcccgaagggagaaaggcggacaggtatccggtaagcggcagggtcggaacaggagagcgcacgagggagcttccagggggaaacgcctggtatctttatagtcctgtcgggtttcgccacctctgacttgagcgtcgatttttgtgatgctcgtcaggggggcggagcctatggaaaaacgccagcaacgcggcctttttacggttcctggccttttgctggccttttgctcacatgttctttcctgcgttatcccctgattctgtggataaccgtattaccgcctttgagtgagctgataccgctcgccgcagccgaacgaccgagcgcagcgagtcagtgagcgaggaagcggaagagcgcccaatacgcaaaccgcctctccccgcgcgttggccgattcattaatgcagcaagctcatggctgactaattttttttatttatgcagaggccgaggccgcctcggcctctgagctattccagaagtagtgaggaggcttttttggaggcctaggcttttgcaaaaagctccccgtggcacgacaggtttcccgactggaaagcgggcagtgagcgcaacgcaattaatgtgagttagctcactcattaggcaccccaggctttacactttatgcttccggctcgtatgttgtgtggaattgtgagcggataacaatttcacacaggaaacagctatgacatgattacgaatttcacaaataaagcatttttttcactgcattctagttgtggtttgtccaaactcatcaatgtatcttatcatgtctggatcaactggataactcaagctaaccaaaatcatcccaaacttcccaccccataccctattaccactgccaattacctgtggtttcatttactctaaacctgtgattcctctgaattattttcattttaaagaaattgtatttgttaaatatgtactacaaacttagtagt

SEQ ID NO: 2 - DNA, 12147 bp, artificial sequence
  artificial vector
tggaagggctaattcactcccaaagaagacaagatatccttgatctgtggatctaccacacacaaggctacttccctgattagcagaactacacaccagggccaggggtcagatatccactgacctttggatggtgctacaagctagtaccagttgagccagataaggtagaagaggccaataaaggagagaacaccagcttgttacaccctgtgagcctgcatgggatggatgacccggagagagaagtgttagagtggaggtttgacagccgcctagcatttcatcacgtggcccgagagctgcatccggagtacttcaagaactgctgatatcgagcttgctacaagggactttccgctggggactttccagggaggcgtggcctgggcgggactggggagtggcgagccctcagatcctgcatataagcagctgctttttgcctgtactgggtctctctggttagaccagatctgagcctgggagctctctggctaactagggaacccactgcttaagcctcaataaagcttgccttgagtgcttcaagtagtgtgtgcccgtctgttgtgtgactctggtaactagagatccctcagacccttttagtcagtgtggaaaatctctagcagtggcgcccgaacagggacttgaaagcgaaagggaaaccagaggagctctctcgacgcaggactcggcttgctgaagcgcgcacggcaagaggcgaggggcggcgactggtgagtacgccaaaaattttgactagcggaggctagaaggagagagatgggtgcgagagcgtcagtattaagcgggggagaattagatcgcgatgggaaaaaattcggttaaggccagggggaaagaaaaaatataaattaaaacatatagtatgggcaagcagggagctagaacgattcgcagttaatcctggcctgttagaaacatcagaaggctgtagacaaatactgggacagctacaaccatcccttcagacaggatcagaagaacttagatcattatataatacagtagcaaccctctattgtgtgcatcaaaggatagagataaaagacaccaaggaagctttagacaagatagaggaagagcaaaacaaaagtaagaccaccgcacagcaagcggccggccgctgatcttcagacctggaggaggagatatgagggacaattggagaagtgaattatataaatataaagtagtaaaaattgaaccattaggagtagcacccaccaaggcaaagagaagagtggtgcagagagaaaaaagagcagtgggaataggagctttgttccttgggttcttgggagcagcaggaagcactatgggcgcagcgtcaatgacgctgacggtacaggccagacaattattgtctggtatagtgcagcagcagaacaatttgctgagggctattgaggcgcaacagcatctgttgcaactcacagtctggggcatcaagcagctccaggcaagaatcctggctgtggaaagatacctaaaggatcaacagctcctggggatttggggttgctctggaaaactcatttgcaccactgctgtgccttggaatgctagttggagtaataaatctctggaacagatttggaatcacacgacctggatggagtgggacagagaaattaacaattacacaagcttaatacactccttaattgaagaatcgcaaaaccagcaagaaaagaatgaacaagaattattggaattagataaatgggcaagtttgtggaattggtttaacataacaaattggctgtggtatataaaattattcataatgatagtaggaggcttggtaggtttaagaatagtttttgctgtactttctatagtgaatagagttaggcagggatattcaccattatcgtttcagacccacctcccaaccccgaggggacccgacaggcccgaaggaatagaagaagaaggtggagagagagacagagacagatccattcgattagtgaacggatctcgacggtatcgccgaattcacaaatggcagtattcatccacaattttaaaagaaaaggggggattggggggtacagtgcaggggaaagaatagtagacataatagcaacagacatacaaactaaagaattacaaaaacaaattacaaaaattcaaaattttcgggtttattacagggacagcagagatccagtttggactagtccacaccctaactgacacactcgagtttaccactccctatcagtgatagagaaaagtgaaagtcgagtttaccactccctatcagtgatagagaaaagtgaaagtcgagtttaccactccctatcagtgatagagaaaagtgaaagtcgagtttaccactccctatcagtgatagagaaaagtgaaagtcgagtttaccactccctatcagtgatagagaaaagtgaaagtcgagtttaccactccctatcagtgatagagaaaagtgaaagtcgagtttaccactccctatcagtgatagagaaaagtgaaagtcgagctcggtacccgggtcgaggtaggcgtgtacggtgggaggcctatataagcagagctcgtttagtgaaccgtcagatcgcctggagacgccatccacgctgttttgacctccatagaagacaccgggaccgatccagcctgcggccgccatggcgaccgcagcgtctaaccactacagcctgctcacctccagcgcctccatcgtgcacgccgagccgcccggcggcatgcagcagggcgcggggggctaccgcgaagcgcagagcctggtgcagggcgactacggcgctctgcagagcaacggacacccgctcagccacgctcaccagtggatcaccgcgctgtcccacggcggcggcggcgggggcggtggcggcggcggggggggcgggggcggcggcgggggcggcggcgacggctccccgtggtccaccagccccctgggccagccggacatcaagccctcggtggtggtgcagcagggcggccgcggagacgagctgcacgggccaggcgccctgcagcagcagcatcagcagcagcaacagcaacagcagcagcaacagcagcaacagcagcagcagcagcagcaacagcggccgccgcatctggtgcaccacgccgctaaccaccacccgggacccggggcatggcggagcgcggcggctgcagcgcacctcccaccctccatgggagcgtccaacggcggcttgctctactcgcagcccagcttcacggtgaacggcatgctgggcgccggcgggcagccggccggtctgcaccaccacggcctgcgggacgcgcacgacgagccacaccatgccgaccaccacccgcacccgcactcgcacccacaccagcagccgccgcccccgccgcccccgcagggtccgcctggccacccaggcgcgcaccacgacccgcactcggacgaggacacgccgacctcggacgacctggagcagttcgccaagcagttcaagcagcggcggatcaaactgggatttacccaagcggacgtggggctggctctgggcaccctgtatggcaacgtgttctcgcagaccaccatctgcaggtttgaggccctgcagctgagcttcaagaacatgtgcaagctgaagcctttgttgaacaagtggttggaggaggcggactcgtcctcgggcagccccacgagcatagacaagatcgcagcgcaagggcgcaagcggaaaaagcggacctccatcgaggtgagcgtcaagggggctctggagagccatttcctcaaatgccccaagccctcggcccaggagatcacctccctcgcggacagcttacagctggagaaggaggtggtgagagtttggttttgtaacaggagacagaaagagaaaaggatgacccctcccggagggactctgccgggcgccgaggatgtgtacggggggagtagggacactccaccacaccacggggtgcagacgcccgtccagggaagtggcgtgaaacagactttgaattttgaccttctcaagttggcgggagacgtggagtccaacccagggcccatggctgtcagcgacgctctgctcccgtccttctccacgttcgcgtccggcccggcgggaagggagaagacactgcgtccagcaggtgccccgactaaccgttggcgtgaggaactctctcacatgaagcgacttcccccacttcccggccgcccctacgacctggcggcgacggtggccacagacctggagagtggcggagctggtgcagcttgcagcagtaacaacccggccctcctagcccggagggagaccgaggagttcaacgacctcctggacctagactttatcctttccaactcgctaacccaccaggaatcggtggccgccaccgtgaccacctcggcgtcagcttcatcctcgtcttccccagcgagcagcggccctgccagcgcgccctccacctgcagcttcagctatccgatccgggccgggggtgacccgggcgtggctgccagcaacacaggtggagggctcctctacagccgagaatctgcgccacctcccacggcccccttcaacctggcggacatcaatgacgtgagcccctcgggcggcttcgtggctgagctcctgcggccggagttggacccagtatacattccgccacagcagcctcagccgccaggtggcgggctgatgggcaagtttgtgctgaaggcgtctctgaccacccctggcagcgagtacagcagcccttcggtcatcagtgttagcaaaggaagcccagacggcagccaccccgtggtagtggcgccctacagcggtggcccgccgcgcatgtgccccaagattaagcaagaggcggtcccgtcctgcacggtcagccggtccctagaggcccatttgagcgctggaccccagctcagcaacggccaccggcccaacacacacgacttccccctggggcggcagctccccaccaggactacccctacactgagtcccgaggaactgctgaacagcagggactgtcaccctggcctgcctcttcccccaggattccatccccatccggggcccaactaccctcctttcctgccagaccagatgcagtcacaagtcccctctctccattatcaagagctcatgccaccgggttcctgcctgccagaggagcccaagccaaagaggggaagaaggtcgtggccccggaaaagaacagccacccacacttgtgactatgcaggctgtggcaaaacctataccaagagttctcatctcaaggcacacctgcgaactcacacaggcgagaaaccttaccactgtgactgggacggctgtgggtggaaattcgcccgctccgatgaactgaccaggcactaccgcaaacacacagggcaccggccctttcagtgccagaagtgtgacagggccttttccaggtcggaccaccttgccttacacatgaagaggcacttttaaagatccctcccccccccctaacgttactggccgaagccgcttggaataaggccggtgtgcgtttgtctatatgttattttccaccatattgccgtcttttggcaatgtgagggcccggaaacctggccctgtcttcttgacgagcattcctaggggtctttcccctctcgccaaaggaatgcaaggtctgttgaatgtcgtgaaggaagcagttcctctggaagcttcttgaagacaaacaacgtctgtagcgaccctttgcaggcagcggaaccccccacctggcgacaggtgcctctgcggccaaaagccacgtgtataagatacacctgcaaaggcggcacaaccccagtgccacgttgtgagttggatagttgtggaaagagtcaaatggctctcctcaagcgtattcaacaaggggctgaaggatgcccagaaggtaccccattgtatgggatctgatctggggcctcggtgcacatgctttacatgtgtttagtcgaggttaaaaaaacgtctaggccccccgaaccacggggacgtggttttcctttgaaaaacacgatgataatatggccacacatatgatgtataacatgatggagacggagctgaagccgccgggcccgcagcaagcttcggggggcggcggcggaggaggcaacgccacggcggcggcgaccggcggcaaccagaagaacagcccggaccgcgtcaagaggcccatgaacgccttcatggtatggtcccgggggcagcggcgtaagatggcccaggagaaccccaagatgcacaactcggagatcagcaagcgcctgggcgcggagtggaaacttttgtccgagaccgagaagcggccgttcatcgacgaggccaagcggctgcgcgctctgcacatgaaggagcacccggattataaataccggccgcggcggaaaaccaagacgctcatgaagaaggataagtacacgcttcccggaggcttgctggcccccggcgggaacagcatggcgagcggggttggggtgggcgccggcctgggtgcgggcgtgaaccagcgcatggacagctacgcgcacatgaacggctggagcaacggcagctacagcatgatgcaggagcagctgggctacccgcagcacccgggcctcaacgctcacggcgcggcacagatgcaaccgatgcaccgctacgacgtcagcgccctgcagtacaactccatgaccagctcgcagacctacatgaacggctcgcccacctacagcatgtcctactcgcagcagggcacccccggtatggcgctgggctccatgggctctgtggtcaagtccgaggccagctccagcccccccgtggttacctcttcctcccactccagggcgccctgccaggccggggacctccgggacatgatcagcatgtacctccccggcgccgaggtgccggagcccgctgcgcccagtagactgcacatggcccagcactaccagagcggcccggtgcccggcacggccattaacggcacactgcccctgtcgcacatgggtagtgggcaatgtactaactacgctttgttgaaactcgctggcgatgttgaaagtaaccccggtcctatgacgatgctcctggacggaggcccgcagttccctgggttgggagtgggcagcttcggtgctccgcgccaccacgagatgcccaaccgcgagcctgcaggcatgggattgaatcccttcggggactcaacccacgctgcggccgccgccgctgccgccgctgccttcaagctgagcccagccaccgctcacgatctgtcttcgggccagagctcagcgttcacaccgcagggttcaggttatgccaatgccctgggccaccatcaccaccaccatcaccaccatcacgccagccaggtgcccacctacggcggcgctgcctccgccgctttcaactccacgcgcgactttctgttccgtcagcgcggttctgggctcagcgaggcagcctccgggggcgggcagcacgggcttttcgctggctcggcgagcagtcttcacgctccagctggtattcctgagcctcctagctacttgctctttcctgggcttcatgagcagggcgctgggcacccgtcgcccacagggcacgtggacaacaaccaggtccatctggggctgcgcggggagctatttggccgtgcagacccataccgccccgtggctagcccgcgcacggacccctacgcggccagtgcgcagttccctaactatagccccatgaacatgaacatgggcgtgaacgtggcggcccaccacgggccgggcgccttcttccgttacatgcggcagcccatcaagcaggagctgtcctgtaagtggatcgaggaggctcagctgagccggcccaagaagagctgcgaccggaccttcagcaccatgcatgagttggttacgcatgttaccatggagcatgtggggggcccggagcagaacaaccacgtctgctattgggaggaatgtccccgcgaaggcaagtccttcaaggcgaagtacaaactggtcaaccatatccgagtgcacactggcgagaaacccttcccgtgtcccttcccgggctgcgggaagatttttgcccgctctgagaacctcaagatccacaagaggacccatacaggtgagaaacctttcaaatgtgaattcgaaggctgtgacagacggtttgccaacagcagcgaccgcaagaagcacatgcatgtgcacacctcggacaagccctatatctgtaaagtgtgcgacaagtcctacacacacccgagctccctgcgcaaacacatgaaggttcatgaatctcaagggtcagattcctcccctgctgccagttcaggctatgaatcttccactccacccgctatagcttctgcaaacagtaaagataccactaaaaccccttctgcagttcaaactagcaccagccacaaccctggacttcctcccaattttaacgaatggtacgtctgaatcgatagatcctaatcaacctctggattacaaaatttgtgaaagattgactggtattcttaactatgttgctccttttacgctatgtggatacgctgctttaatgcctttgtatcatgctattgcttcccgtatggctttcattttctcctccttgtataaatcctggttgctgtctctttatgaggagttgtggcccgttgtcaggcaacgtggcgtggtgtgcactgtgtttgctgacgcaacccccactggttggggcattgccaccacctgtcagctcctttccgggactttcgctttccccctccctattgccacggcggaactcatcgccgcctgccttgcccgctgctggacaggggctcggctgttgggcactgacaattccgtggtgttgtcggggaaatcatcgtcctttccttggctgctcgcctgtgttgccacctggattctgcgcgggacgtccttctgctacgtcccttcggccctcaatccagcggaccttccttcccgcggcctgctgccggctctgcggcctcttccgcgtcttcgccttcgccctcagacgagtcggatctccctttgggccgcctccccgcctggtacctttaagaccaatgacttacaaggcagctgtagatcttagccactttttaaaagaaaaggggggactggaagggctaattcactcccaacgaagacaagatcacctgcaggacaggcgcgccataacttcgtatagcatacattatacgaagttatggtacctgcgcgccctgctttttgcttgtactgggtctctctggttagaccagatctgagcctgggagctctctggctaactagggaacccactgcttaagcctcaataaagcttgccttgagtgcttcaagtagtgtgtgcccgtctgttgtgtgactctggtaactagagatccctcagacccttttagtcagtgtggaaaatctctagcacccgggcgattaaggaaagggctagatcattcttgaagacgaaagggcctcgtgatacgcctatttttataggttaatgtcatgataataatggtttcttagacgtcaggtggcacttttcggggaaatgtgcgcggaacccctatttgtttatttttctaaatacattcaaatatgtatccgctcatgagacaataaccctgataaatgcttcaataatattgaaaaaggaagagtatgagtattcaacatttccgtgtcgcccttattcccttttttgcggcattttgccttcctgtttttgctcacccagaaacgctggtgaaagtaaaagatgctgaagatcagttgggtgcacgagtgggttacatcgaactggatctcaacagcggtaagatccttgagagttttcgccccgaagaacgttttccaatgatgagcacttttaaagttctgctatgtggcgcggtattatcccgtgttgacgccgggcaagagcaactcggtcgccgcatacactattctcagaatgacttggttgagtactcaccagtcacagaaaagcatcttacggatggcatgacagtaagagaattatgcagtgctgccataaccatgagtgataacactgcggccaacttacttctgacaacgatcggaggaccgaaggagctaaccgcttttttgcacaacatgggggatcatgtaactcgccttgatcgttgggaaccggagctgaatgaagccataccaaacgacgagcgtgacaccacgatgcctgtagcaatggcaacaacgttgcgcaaactattaactggcgaactacttactctagcttcccggcaacaattaatagactggatggaggcggataaagttgcaggaccacttctgcgctcggcccttccggctggctggtttattgctgataaatctggagccggtgagcgtgggtctcgcggtatcattgcagcactggggccagatggtaagccctcccgtatcgtagttatctacacgacggggagtcaggcaactatggatgaacgaaatagacagatcgctgagataggtgcctcactgattaagcattggtaactgtcagaccaagtttactcatatatactttagattgatttaaaacttcatttttaatttaaaaggatctaggtgaagatcctttttgataatctcatgaccaaaatcccttaacgtgagttttcgttccactgagcgtcagaccccgtagaaaagatcaaaggatcttcttgagatcctttttttctgcgcgtaatctgctgcttgcaaacaaaaaaaccaccgctaccagcggtggtttgtttgccggatcaagagctaccaactctttttccgaaggtaactggcttcagcagagcgcagataccaaatactgttcttctagtgtagccgtagttaggccaccacttcaagaactctgtagcaccgcctacatacctcgctctgctaatcctgttaccagtggctgctgccagtggcgataagtcgtgtcttaccgggttggactcaagacgatagttaccggataaggcgcagcggtcgggctgaacggggggttcgtgcacacagcccagcttggagcgaacgacctacaccgaactgagatacctacagcgtgagctatgagaaagcgccacgcttcccgaagggagaaaggcggacaggtatccggtaagcggcagggtcggaacaggagagcgcacgagggagcttccagggggaaacgcctggtatctttatagtcctgtcgggtttcgccacctctgacttgagcgtcgatttttgtgatgctcgtcaggggggcggagcctatggaaaaacgccagcaacgcggcctttttacggttcctggccttttgctggccttttgctcacatgttctttcctgcgttatcccctgattctgtggataaccgtattaccgcctttgagtgagctgataccgctcgccgcagccgaacgaccgagcgcagcgagtcagtgagcgaggaagcggaagagcgcccaatacgcaaaccgcctctccccgcgcgttggccgattcattaatgcagcaagctcatggctgactaattttttttatttatgcagaggccgaggccgcctcggcctctgagctattccagaagtagtgaggaggcttttttggaggcctaggcttttgcaaaaagctccccgtggcacgacaggtttcccgactggaaagcgggcagtgagcgcaacgcaattaatgtgagttagctcactcattaggcaccccaggctttacactttatgcttccggctcgtatgttgtgtggaattgtgagcggataacaatttcacacaggaaacagctatgacatgattacgaatttcacaaataaagcatttttttcactgcattctagttgtggtttgtccaaactcatcaatgtatcttatcatgtctggatcaactggataactcaagctaaccaaaatcatcccaaacttcccaccccataccctattaccactgccaattacctgtggtttcatttactctaaacctgtgattcctctgaattattttcattttaaagaaattgtatttgttaaatatgtactacaaacttagtagt

SEQ ID NO: 3 - DNA, 20 bp, artificial sequence
  artificial primer sequence
ctggagaaggaggtggtgag

SEQ ID NO: 4 - DNA, 19 bp, artificial sequence
  artificial primer sequence
gagaaggacgggagcagag

SEQ ID NO: 5 - DNA, 19 bp, artificial sequence
  artificial primer sequence
cctgtcgcacatgggtagt

SEQ ID NO: 6 - DNA, 20 bp, artificial sequence
  artificial primer sequence
gattcaatcccatgcctgca

SEQ ID NO: 7 - DNA, 20 bp, artificial sequence
  artificial primer sequence
gcctcccagtggtatttgaa

SEQ ID NO: 8 - DNA, 20 bp, artificial sequence
  artificial primer sequence
agcaggtaaccggaaccttt

SEQ ID NO: 9 - DNA, 21 bp, artificial sequence
  artificial primer sequence
acctcgaagtacaaggtcacg

SEQ ID NO: 10 - DNA, 25 bp, artificial sequence
  artificial primer sequence
gatcttcctccatttttagacttcg

SEQ ID NO: 11 - DNA, 21 bp, artificial sequence
  artificial primer sequence
ccagaaaggatgcctcataaa

SEQ ID NO: 12 - DNA, 18 bp, artificial sequence
  artificial primer sequence
tctgcgcgcccctagtta

SEQ ID NO: 13 - DNA, 25 bp, artificial sequence
  artificial primer sequence
agagatcacctcttgcttgagaacg

SEQ ID NO: 14 - DNA, 22 bp, artificial sequence
  artificial primer sequence
ggagcctgtgctgtagcaatca

SEQ ID NO: 15 - DNA, 19 bp, artificial sequence
  artificial primer sequence
acccctgcctaaccacatc

SEQ ID NO: 16 - DNA, 21 bp, artificial sequence
  artificial primer sequence
gcggcaaagaatcttggagac

SEQ ID NO: 17 - DNA, 20 bp, artificial sequence
  artificial primer sequence
tggcgaaccatctctgtggt

SEQ ID NO: 18 - DNA, 20 bp, artificial sequence
  artificial primer sequence
ccaacggtgtcaacctgcat

SEQ ID NO: 19 - DNA, 20 bp, artificial sequence
  artificial primer sequence
aggtccatgtggagcttgac

SEQ ID NO: 20 - DNA, 20 bp, artificial sequence
  artificial primer sequence
gccattgcctcatactgcgt

SEQ ID NO: 21 - DNA, 19 bp, artificial sequence
  artificial primer sequence
ggctttgccactaggcagg

SEQ ID NO: 22 - DNA, 23 bp, artificial sequence
  artificial primer sequence
tgaccactttgtctccttcttga

SEQ ID NO: 23 - DNA, 20 bp, artificial sequence
  artificial primer sequence
tgcgagcagagagggagtag

SEQ ID NO: 24 - DNA, 22 bp, artificial sequence
  artificial primer sequence
tgagttccatgaaggcaggatg

SEQ ID NO: 25 - DNA, 20 bp, artificial sequence
  artificial primer sequence
aaccgctacatcacggagca

SEQ ID NO: 26 - DNA, 20 bp, artificial sequence
  artificial primer sequence
gatcttggcgcgcttgttct

SEQ ID NO: 27 - DNA, 20 bp, artificial sequence
  artificial primer sequence
gcagagcagcaggaagctga

SEQ ID NO: 28 - DNA, 21 bp, artificial sequence
  artificial primer sequence
ttctgccgaggaggctaagtg

SEQ ID NO: 29 - DNA, 21 bp, artificial sequence
  artificial primer sequence
tgcttcaggagcagcaaacaa

SEQ ID NO: 30 - DNA, 20 bp, artificial sequence
  artificial primer sequence
gatccaacgcccttccagag

SEQ ID NO: 31 - DNA, 20 bp, artificial sequence
  artificial primer sequence
aagcagccggagaagaccac

SEQ ID NO: 32 - DNA, 20 bp, artificial sequence
  artificial primer sequence
tccttcatgagcgcatctgg

SEQ ID NO: 33 - DNA, 20 bp, artificial sequence
  artificial primer sequence
ggtggaggaagctgacaaca

SEQ ID NO: 34 - DNA, 20 bp, artificial sequence
  artificial primer sequence
atctgctgcagtgtgggttt

SEQ ID NO: 35 - DNA, 21 bp, artificial sequence
  artificial primer sequence
cagcagtgtcgctccaattca

SEQ ID NO: 36 - DNA, 20 bp, artificial sequence
  artificial primer sequence
gccaagcaccgaattcacag

SEQ ID NO: 37 - DNA, 19 bp, artificial sequence
  artificial primer sequence
cgttcggagcactatgctg

SEQ ID NO: 38 - DNA, 21 bp, artificial sequence
  artificial primer sequence
tgttgcacgactttttggggt

SEQ ID NO: 39 - DNA, 21 bp, artificial sequence
  artificial primer sequence
ggcgctcagtttcctaactac

SEQ ID NO: 40 - DNA, 21 bp, artificial sequence
  artificial primer sequence
ctgccgcatataacggaagaa

SEQ ID NO: 41 - DNA, 20 bp, artificial sequence
  artificial primer sequence
agacgcaggtgaaggtgtgg

SEQ ID NO: 42 - DNA, 18 bp, artificial sequence
  artificial primer sequence
caggcaggcaggctctcc

SEQ ID NO: 43 - DNA, 24 bp, artificial sequence
  artificial primer sequence
tgggagataggaaagaggtgaaaa

SEQ ID NO: 44 - DNA, 19 bp, artificial sequence
  artificial primer sequence
gcaccaggctgttgatgct

SEQ ID NO: 45 - DNA, 23 bp, artificial sequence
  artificial primer sequence
caaagtgagacctgccaaaaaga

SEQ ID NO: 46 - DNA, 21 bp, artificial sequence
  artificial primer sequence
tggacaagggatctgacagtg

SEQ ID NO: 47 - DNA, 20 bp, artificial sequence
  artificial primer sequence
ccgccttcagcatagactcg

SEQ ID NO: 48 - DNA, 21 bp, artificial sequence
  artificial primer sequence
ggtagccggtgtagacgaaat

SEQ ID NO: 49 - DNA, 19 bp, artificial sequence
  artificial primer sequence
cctgggacccatttcggac

SEQ ID NO: 50 - DNA, 19 bp, artificial sequence
  artificial primer sequence
tggagccagactcaggacc

SEQ ID NO: 51 - DNA, 20 bp, artificial sequence
  artificial primer sequence
ctctgcttccaaaggtgtcc

SEQ ID NO: 52 - DNA, 18 bp, artificial sequence
  artificial primer sequence
caggtcctggccaacaag

SEQ ID NO: 53 - DNA, 23 bp, artificial sequence
  artificial primer sequence
tcaagtcgagtctatctgcatcc

SEQ ID NO: 54 - DNA, 21 bp, artificial sequence
  artificial primer sequence
catgtcacgaccagtcacaac

SEQ ID NO: 55 - DNA, 20 bp, artificial sequence
  artificial primer sequence
gctcgctgagtgcctgacat

SEQ ID NO: 56 - DNA, 23 bp, artificial sequence
  artificial primer sequence
ggaggaggaatcagtgtcgagtg

SEQ ID NO: 57 - DNA, 20 bp, artificial sequence
  artificial primer sequence
tttagccgttcgcttagagg

SEQ ID NO: 58 - DNA, 20 bp, artificial sequence
  artificial primer sequence
cggatagctggagacaggag

SEQ ID NO: 59 - DNA, 20 bp, artificial sequence
  artificial primer sequence
gcctcggagaacgaggaaga

SEQ ID NO: 60 - DNA, 20 bp, artificial sequence
  artificial primer sequence
cgctgctggacttgtgcttc

SEQ ID NO: 61 - DNA, 24 bp, artificial sequence
  artificial primer sequence
gacaactggtggcagatttcgctt

SEQ ID NO: 62 - DNA, 24 bp, artificial sequence
  artificial primer sequence
agccacaaagaaaggagttggacc

SEQ ID NO: 63 - DNA, 19 bp, artificial sequence
  artificial primer sequence
agcagggagtccgtaaacg

SEQ ID NO: 64 - DNA, 23 bp, artificial sequence
  artificial primer sequence
agcattccgaaacaggtaacttt

SEQ ID NO: 65 - DNA, 20 bp, artificial sequence
  artificial primer sequence
gactagagtctgagatgccc

SEQ ID NO: 66 - DNA, 20 bp, artificial sequence
  artificial primer sequence
agacattgttaaattgcccg

SEQ ID NO: 67 - DNA, 19 bp, artificial sequence
  artificial primer sequence
agcgaacgcacatcaagac

SEQ ID NO: 68 - DNA, 20 bp, artificial sequence
  artificial primer sequence
ctgtaggcgatctgttgggg

SEQ ID NO: 69 - DNA, 19 bp, artificial sequence
  artificial primer sequence
ctgggctacactgagcacc

SEQ ID NO: 70 - DNA, 21 bp, artificial sequence
  artificial primer sequence
aagtggtcgttgagggcaatg

SEQ ID NO: 71 - DNA, 24 bp, artificial sequence
  artificial primer sequence
cgagaggaccccgtggatgcagag

SEQ ID NO: 72 - DNA, 24 bp, artificial sequence
  artificial primer sequence
ggcggccatcttcagcttctccag

SEQ ID NO: 73 - DNA, 23 bp, artificial sequence
  artificial primer sequence
tttcagctagcatcctgtactcc

SEQ ID NO: 74 - DNA, 21 bp, artificial sequence
  artificial primer sequence
gaccctggtcttgtcgttaga

SEQ ID NO: 75 - DNA, 21 bp, artificial sequence
  artificial primer sequence
cccattctcggccttgactgt

SEQ ID NO: 76 - DNA, 23 bp, artificial sequence
  artificial primer sequence
gtggagattgttgccatcaacga

SEQ ID NO: 77 - DNA, 22 bp, artificial sequence
  artificial primer sequence
cggaggacaaaagacaaaaacc

SEQ ID NO: 78 - DNA, 21 bp, artificial sequence
  artificial primer sequence
aagttacagagccggcagtca

SEQ ID NO: 79 - DNA, 26 bp, artificial sequence
  artificial primer sequence
atgggcattggtatgttataatgaag

SEQ ID NO: 80 - DNA, 19 bp, artificial sequence
  artificial primer sequence
aacacagatccgcgatcca

SEQ ID NO: 81 - DNA, 21 bp, artificial sequence
  artificial primer sequence
tgctgctatgacttctttgcc

SEQ ID NO: 82 - DNA, 19 bp, artificial sequence
  artificial primer sequence
gcttcctgtgatcggccat

SEQ ID NO: 83 - DNA, 19 bp, artificial sequence
  artificial primer sequence
ccggggcagaattacccac

SEQ ID NO: 84 - DNA, 22 bp, artificial sequence
  artificial primer sequence
gccgttgataaatactcctccg

SEQ ID NO: 85 - DNA, 17 bp, artificial sequence
  artificial primer sequence
tcccccgccaaacttca

SEQ ID NO: 86 - DNA, 20 bp, artificial sequence
  artificial primer sequence
gtaccacccatcccttcgaa

SEQ ID NO: 87 - DNA, 20 bp, artificial sequence
  artificial primer sequence
tgcaggatccctacgccaac

SEQ ID NO: 88 - DNA, 22 bp, artificial sequence
  artificial primer sequence
cctgatgctggagcctgttctt

SEQ ID NO: 89 - DNA, 21 bp, artificial sequence
  artificial primer sequence
tctgggtccctatccaatgtg

SEQ ID NO: 90 - DNA, 19 bp, artificial sequence
  artificial primer sequence
ggtccccgaactggtactg

SEQ ID NO: 91 - DNA, 21 bp, artificial sequence
  artificial primer sequence
ccgaggagggatctaaggaac

SEQ ID NO: 92 - DNA, 23 bp, artificial sequence
  artificial primer sequence
cttccaaaagtatcggtctccac

SEQ ID NO: 93 - DNA, 20 bp, artificial sequence
  artificial primer sequence
cagcgaccaccttcccatac

SEQ ID NO: 94 - DNA, 22 bp, artificial sequence
  artificial primer sequence
cgcagtgtttgtccttgtgtct

SEQ ID NO: 95 - DNA, 20 bp, artificial sequence
  artificial primer sequence
tgcctcggccacaaagaatc

SEQ ID NO: 96 - DNA, 20 bp, artificial sequence
  artificial primer sequence
gttggtgtacgcggttctca

SEQ ID NO: 97 - DNA, 22 bp, artificial sequence
  artificial primer sequence
accaagaaacccagccaatccg

SEQ ID NO: 98 - DNA, 19 bp, artificial sequence
  artificial primer sequence
gcaatccggggccatctga

SEQ ID NO: 99 - DNA, 23 bp, artificial sequence
  artificial primer sequence
atgggggaatctttaatgctggt

SEQ ID NO: 100 - DNA, 22 bp, artificial sequence
  artificial primer sequence
agcactcatgaaatgggacact

SEQ ID NO: 101 - DNA, 23 bp, Homo sapiens
ccaaatcgttccgaatgttttgc

SEQ ID NO: 102 - DNA, 61 bp, Homo sapiens
cggtttcctgcaagtcaagttccaaatcgttccgaatgttttgcccttatgaatgttagtc

SEQ ID NO: 103 - DNA, 51 bp, Homo sapiens
cggtttcctgcaagtcaagttccaaatgttttgcccttatgaatgttagtc

SEQ ID NO: 104 - DNA, 56 bp, Homo sapiens
cggtttcctgcaagtcaagttccaaatcgaatgttttgcccttatgaatgttagtc

SEQ ID NO: 105 - DNA, 51 bp, Homo sapiens
cggtttcctgcaagtcaagttccgaatgttttgcccttatgaatgttagtc